European Patent Specification EP 4 627 105 B1, published June 10, 2026. Title: Method for identifying a modified amino acid degron (MAAD). Applicant: ETH Zuerich. Application EP. The sequence listing filed with the application follows.

SEQUENCE LISTING (40 sequences)

SEQ ID NO: 1 - protein, 5 aa, synthetic construct
  VARIANT 3: note = X is any natural amino acid
LPXTG

SEQ ID NO: 2 - protein, 6 aa, synthetic construct
LPETGG

SEQ ID NO: 3 - protein, 5 aa, synthetic construct
NPQTN

SEQ ID NO: 4 - protein, 5 aa, synthetic construct
NPKTG

SEQ ID NO: 5 - protein, 6 aa, synthetic construct
GSGSGS

SEQ ID NO: 6 - protein, 8 aa, synthetic construct
GSGSGSGS

SEQ ID NO: 7 - protein, 5 aa, synthetic construct
GGGGG

SEQ ID NO: 8 - protein, 33 aa, synthetic construct
  VARIANT 13: note = L-Dopa
  VARIANT 18: note = L-Dopa
GGGKDLEGKGGSXGSGSXGGSKYPYDVPDYAKD

SEQ ID NO: 9 - protein, 33 aa, synthetic construct; identical to SEQ ID NO: 8
  VARIANT 13: note = Hexanoyllysine
  VARIANT 17: note = Hexanoyllysine

SEQ ID NO: 10 - protein, 33 aa, synthetic construct; identical to SEQ ID NO: 8
  VARIANT 13: note = Carboxymethyllysine
  VARIANT 17: note = Carboxymethyllysine

SEQ ID NO: 11 - protein, 33 aa, synthetic construct; identical to SEQ ID NO: 8
  VARIANT 13: note = Homocitrulline
  VARIANT 17: note = Homocitrulline

SEQ ID NO: 12 - protein, 33 aa, synthetic construct
GGGKDLEGKGGSAGSGSAGGSKYPYDVPDYAKD

SEQ ID NO: 13 - protein, 33 aa, synthetic construct
GGGKDLEGKGGSYGSGSYGGSKYPYDVPDYAKD

SEQ ID NO: 14 - protein, 33 aa, synthetic construct; identical to SEQ ID NO: 12
  MOD_RES 33: note = Amidation

SEQ ID NO: 15 - protein, 33 aa, synthetic construct
GGGKDLEGKGGSAGSGSAGGSKYPYDVPDYAKS

SEQ ID NO: 16 - protein, 33 aa, synthetic construct; identical to SEQ ID NO: 15
  MOD_RES 33: note = amidation

SEQ ID NO: 17 - protein, 26 aa, synthetic construct
GGGRRLEGKEEDEKGSRASDRFRGLR

SEQ ID NO: 18 - protein, 26 aa, synthetic construct
GGGRRLEGKEEDEKGSRASDDFRDLR

SEQ ID NO: 19 - protein, 26 aa, synthetic construct
  MOD_RES 26: note = amidation
GGGRRLEGKEEDEKGSRASDDFRDLR

SEQ ID NO: 20 - protein, 253 aa, Entacmaea quadricolor
MVSKGEELIKENMHMKLYMEGTVDNHHFKCTSEGEGKPYEGTQTMRIKVVEGGPLPFAFDILATSFLYGSKTFINHTQGIPDFFKQSFPEGFTWERVTTYEDGGVLTATQDTSLQDGCLIYNVKIRGVNFTSNGPVMQKKTLGWEAFTETLYPADGGLEGRNDMALKLVGGSHLIANAKTTYRSKKPAKNLKMPGVYYVDYRLERIKEANNETYVEQHEVAVARYCDLPSKLGHKLNSGGLPETGGHHHHHHV

SEQ ID NO: 21 - protein, 256 aa, Aequorea victoria
MSMSKGEELFTGVVPILVELDGDVNGHKFSVRGEGEGDATNGKLTLKFICTTGKLPVPWPTLVTTLTYGVQCFARYPDHMKQHDFFKSAMPEGYVQERTISFKDDGTYKTRAEVKFEGDTLVNRIELKGIDFKEDGNILGHKLEYNFNSHNVYITADKQKNGIKANFKIRHNVEDGSVQLADHYQQNTPIGDGPVLLPDNHYLSTQSKLSKDPNEKRDHMVLLEFVTAAGITHGMDELYKSGGLPETGGHHHHHHV

SEQ ID NO: 22 - protein, 252 aa, Discosoma sp.
MVSKGEEDNMAIIKEFMRFKVHMEGSVNGHEFEIEGEGEGRPYEGTQTAKLKVTKGGPLPFAWDILSPQFMYGSKAYVKHPADIPDYLKLSFPEGFKWERVMNFEDGGVVTVTQDSSLQDGEFIYKVKLRGTNFPSDGPVMQKKTMGWEASSERMYPEDGALKGEIKQRLKLKDGGHYDAEVKTTYKAKKPVQLPGAYNVNIKLDITSHNEDYTIVEQYERAEGRHSTGGMDELYKSGGLPETGGHHHHHHV

SEQ ID NO: 23 - protein, 273 aa, synthetic construct
MSMSKGEELFTGVVPILVELDGDVNGHKFSVRGEGEGDATNGKLTLKFICTTGKLPVPWPTLVTTLTYGVQCFARYPDHMKQHDFFKSAMPEGYVQERTISFKDDGTYKTRAEVKFEGDTLVNRIELKGIDFKEDGNILGHKLEYNFNSHNVYITADKQKNGIKANFKIRHNVEDGSVQLADHYQQNTPIGDGPVLLPDNHYLSTQSKLSKDPNEKRDHMVLLEFVTAAGITHGMDELYKSGGLPETGGGRRLEGKEEDEKGSRASDRFRGLR

SEQ ID NO: 24 - protein, 273 aa, synthetic construct
MSMSKGEELFTGVVPILVELDGDVNGHKFSVRGEGEGDATNGKLTLKFICTTGKLPVPWPTLVTTLTYGVQCFARYPDHMKQHDFFKSAMPEGYVQERTISFKDDGTYKTRAEVKFEGDTLVNRIELKGIDFKEDGNILGHKLEYNFNSHNVYITADKQKNGIKANFKIRHNVEDGSVQLADHYQQNTPIGDGPVLLPDNHYLSTQSKLSKDPNEKRDHMVLLEFVTAAGITHGMDELYKSGGLPETGGGRRLEGKEEDEKGSRASDDFRDLR

SEQ ID NO: 25 - protein, 273 aa, synthetic construct; identical to SEQ ID NO: 24
  MOD_RES 273: note = amidation

SEQ ID NO: 26 - protein, 280 aa, synthetic construct
  MOD_RES 280: note = amidation
MSMSKGEELFTGVVPILVELDGDVNGHKFSVRGEGEGDATNGKLTLKFICTTGKLPVPWPTLVTTLTYGVQCFARYPDHMKQHDFFKSAMPEGYVQERTISFKDDGTYKTRAEVKFEGDTLVNRIELKGIDFKEDGNILGHKLEYNFNSHNVYITADKQKNGIKANFKIRHNVEDGSVQLADHYQQNTPIGDGPVLLPDNHYLSTQSKLSKDPNEKRDHMVLLEFVTAAGITHGMDELYKSGGLPETGGGKDLEGKGGSAGSGSAGGSKYPYDVPDYAKS

SEQ ID NO: 27 - protein, 270 aa, synthetic construct
MVSKGEELIKENMHMKLYMEGTVDNHHFKCTSEGEGKPYEGTQTMRIKVVEGGPLPFAFDILATSFLYGSKTFINHTQGIPDFFKQSFPEGFTWERVTTYEDGGVLTATQDTSLQDGCLIYNVKIRGVNFTSNGPVMQKKTLGWEAFTETLYPADGGLEGRNDMALKLVGGSHLIANAKTTYRSKKPAKNLKMPGVYYVDYRLERIKEANNETYVEQHEVAVARYCDLPSKLGHKLNSGGLPETGGGRRLEGKEEDEKGSRASDRFRGLR

SEQ ID NO: 28 - protein, 270 aa, synthetic construct
MVSKGEELIKENMHMKLYMEGTVDNHHFKCTSEGEGKPYEGTQTMRIKVVEGGPLPFAFDILATSFLYGSKTFINHTQGIPDFFKQSFPEGFTWERVTTYEDGGVLTATQDTSLQDGCLIYNVKIRGVNFTSNGPVMQKKTLGWEAFTETLYPADGGLEGRNDMALKLVGGSHLIANAKTTYRSKKPAKNLKMPGVYYVDYRLERIKEANNETYVEQHEVAVARYCDLPSKLGHKLNSGGLPETGGGRRLEGKEEDEKGSRASDDFRDLR

SEQ ID NO: 29 - protein, 270 aa, synthetic construct; identical to SEQ ID NO: 28
  MOD_RES 270: note = amidation

SEQ ID NO: 30 - protein, 269 aa, synthetic construct
MVSKGEEDNMAIIKEFMRFKVHMEGSVNGHEFEIEGEGEGRPYEGTQTAKLKVTKGGPLPFAWDILSPQFMYGSKAYVKHPADIPDYLKLSFPEGFKWERVMNFEDGGVVTVTQDSSLQDGEFIYKVKLRGTNFPSDGPVMQKKTMGWEASSERMYPEDGALKGEIKQRLKLKDGGHYDAEVKTTYKAKKPVQLPGAYNVNIKLDITSHNEDYTIVEQYERAEGRHSTGGMDELYKSGGLPETGGGRRLEGKEEDEKGSRASDRFRGLR

SEQ ID NO: 31 - protein, 269 aa, synthetic construct
MVSKGEEDNMAIIKEFMRFKVHMEGSVNGHEFEIEGEGEGRPYEGTQTAKLKVTKGGPLPFAWDILSPQFMYGSKAYVKHPADIPDYLKLSFPEGFKWERVMNFEDGGVVTVTQDSSLQDGEFIYKVKLRGTNFPSDGPVMQKKTMGWEASSERMYPEDGALKGEIKQRLKLKDGGHYDAEVKTTYKAKKPVQLPGAYNVNIKLDITSHNEDYTIVEQYERAEGRHSTGGMDELYKSGGLPETGGGRRLEGKEEDEKGSRASDDFRDLR

SEQ ID NO: 32 - protein, 269 aa, synthetic construct; identical to SEQ ID NO: 31
  MOD_RES 268: note = amidation

SEQ ID NO: 33 - DNA, 22 bp, Homo sapiens
  source 1..22: mol_type = genomic DNA
gagggcctatttcccatgattc

SEQ ID NO: 34 - DNA, 22 bp, Homo sapiens
  source 1..22: mol_type = genomic DNA
caaacccagggctgccttggaa

SEQ ID NO: 35 - DNA, 70 bp, synthetic construct
  source 1..70: mol_type = other DNA
aatgatacggcgaccaccgagatctacacgagaggttacactctttccctacacgacgctcttccgatct

SEQ ID NO: 36 - DNA, 65 bp, synthetic construct
  source 1..65: mol_type = other DNA
caagcagaagacggcatacgagatggatctgagtgactggagttcagacgtgtgctcttccgatc

SEQ ID NO: 37 - DNA, 92 bp, synthetic construct
  source 1..92: mol_type = other DNA
aatgatacggcgaccaccgagatctacacgatatcgaacactctttccctacacgacgctcttccgatctttgtggaaaggacgaggtaccg

SEQ ID NO: 38 - DNA, 92 bp, synthetic construct
  source 1..92: mol_type = other DNA
aatgatacggcgaccaccgagatctacaccgcagacgacactctttccctacacgacgctcttccgatctttgtggaaaggacgaggtaccg

SEQ ID NO: 39 - DNA, 90 bp, synthetic construct
  source 1..90: mol_type = other DNA
caagcagaagacggcatacgagatccgcggttgtgactggagttcagacgtgtgctcttccgatctacttgctatttctagctctaaaac

SEQ ID NO: 40 - DNA, 90 bp, synthetic construct
  source 1..90: mol_type = other DNA
caagcagaagacggcatacgagataagtccaagtgactggagttcagacgtgtgctcttccgatctacttgctatttctagctctaaaac